European Patent Application EP 4 640 708 A1, published October 29, 2025. Title: NOVEL ANTI-GPRC5D ANTIBODY. Applicant: CHIMAGEN BIOSCIENCES, LTD. The sequence listing filed with the application follows.

SEQUENCE LISTING (27 sequences)

SEQ ID NO: 1 - protein, 5 aa, synthetic
SSVSF

SEQ ID NO: 2 - skipped

SEQ ID NO: 3 - protein, 9 aa, synthetic
QQWNSHPLT

SEQ ID NO: 4 - protein, 8 aa, synthetic
GYPFTNYW

SEQ ID NO: 5 - protein, 8 aa, synthetic
INPSNGRT

SEQ ID NO: 6 - protein, 6 aa, synthetic
ARGFAY

SEQ ID NO: 7 - protein, 10 aa, synthetic
SASSSVSFMH

SEQ ID NO: 8 - protein, 7 aa, synthetic
DTTKLAS

SEQ ID NO: 9 - protein, 5 aa, synthetic
NYWMH

SEQ ID NO: 10 - protein, 17 aa, synthetic
EINPSNGRTNYNEKFKS

SEQ ID NO: 11 - protein, 4 aa, synthetic
GFAY

SEQ ID NO: 12 - protein, 106 aa, synthetic
QIVLSQFPAIMSASPGEKVTMTCSASSSVSFMHWYQQKSGTSPKRWIYDTTKLASGVPARFTGSGSGTSYSLTISSMEAEDAATYYCQQWNSHPLTFGPGTKLELK

SEQ ID NO: 13 - protein, 113 aa, synthetic
QVQLQQPGAELVKPGTSVKLSCKASGYPFTNYWMHWVRQRPGQGLEWIGEINPSNGRTNYNEKFKSLATLTLDKSSSTAYMHLNSLTSEDSAVYYCARGFAYWGQGTLVTVSA

SEQ ID NO: 14 - protein, 106 aa, synthetic
EIVLTQSPGTLSLSPGERATLSCSASSSVSFMHWYQQKPGQAPRRWIYDTTKLASGIPDRFSGSGSGTDYTLTISRLEPEDFAVYYCQQWNSHPLTFGQGTTVEIK

SEQ ID NO: 15 - protein, 113 aa, synthetic
QVQLVQSGAEVKKPGSSVKVSCRASGYPFTNYWMHWVRQAPGQGLEWIGEINPSNGRTNYNEKFKSRATLTLDKLTSTAYMELSSLTSEDTALYYCARGFAYWGQGTLVTVSS

SEQ ID NO: 16 - protein, 106 aa, synthetic
EIVLTQSPATLSLSPGERATLSCSASSSVSFMHWYQQKPGQAPRRWIYDTTKLASGIPARFSGSGSGTDYTLTISSLEPEDFAVYYCQQWNSHPLTFGQGTKLEIK

SEQ ID NO: 17 - protein, 113 aa, synthetic
EVTLKESGPVLVKPTETLTLTCTASGYPFTNYWMHWVRQPPGKALEWIGEINPSNGRTNYNEKFKSRATLSLDKSKSQAVLTMTNMDPVDTATYYCARGFAYWGQGTLVTVSS

SEQ ID NO: 18 - protein, 106 aa, synthetic
EIVLTQSPATLSLSPGERATLSCSASSSVSFMHWYQQKPGQAPRRWIYDTTKLASGVPARFSGSGSGTDYTLTISSLEPEDFAVYYCQQWNSHPLTFGQGTKVEIK

SEQ ID NO: 19 - protein, 111 aa, synthetic
ELVQSGAEVKKPGSSVKVSCKASGYPFTNYWMHWVRQAPGQGLEWIGEINPSNGRTNYNEKFKSRATLTLDKSTSTAYMELSSLRSEDTAVYYCARGFAYWGQGTLVTVSS

SEQ ID NO: 20 - protein, 106 aa, synthetic
AIQLTQSPSSLSASVGDRVTITCSASSSVSFMHWYQQKPGKAPKRWIYDTTKLASGVPSRFSGSGSGTDYTFTISSLQPEDIATYYCQQWNSHPLTFGPGTKVDIK

SEQ ID NO: 21 - protein, 113 aa, synthetic
QVQLQESGPGLVKPSETLSLTCTASGYPFTNYWMHWVRQPPGKGLEWIGEINPSNGRTNYNEKFKSRATLSLDKSKNQASLNLDSVSAADTAIYYCARGFAYWGKGSTVTVSS

SEQ ID NO: 22 - protein, 445 aa, synthetic
QVQLVQSGAEVKKPGASVKVSCKASGYSFTGYTMNWVRQAPGQGLEWMGLINPYNSDTNYAQKLQGRVTMTTDTSTSTAYMELRSLRSDDTAVYYCARVALRVALDYWGQGTLVTVSSASTKGPSVFPLAPCSRSTSESTAALGCLVKDYFPEPVTVSWNSGALTSGVHTFPAVLQSSGLYSLSSVVTVPSSSLGTKTYTCNVDHKPSNTKVDKRVESKYGPPCPPCPAPEFLGGPSVFLFPPKPKDTLMISRTPEVTCVVVDVSQEDPEVQFNWYVDGVEVHNAKTKPREEQFNSTYRVVSVLTVLHQDWLNGKEYKCKVSNKGLPSSIEKTISKAKGQPREPQVYTLPPSQEEMTKNQVSLTCLVKGFYPSDIAVEWESNGQPENNYKTTPPVLDSDGSFFLYSRLTVDKSRWQEGNVFSCSVMHEALHNHYTQKSLSLSLGK

SEQ ID NO: 23 - protein, 214 aa, synthetic
DIQMTQSPSSLSASVGDRVTITCKASQNVATHVGWYQQKPGKAPKRLIYSASYRYSGVPSRFSGSGSGTEFTLTISNLQPEDFATYYCQQYNRYPYTFGQGTKLEIKRTVAAPSVFIFPPSDEQLKSGTASVVCLLNNFYPREAKVQWKVDNALQSGNSQESVTEQDSKDSTYSLSSTLTLSKADYEKHKVYACEVTHQGLSSPVTKSFNRGEC

SEQ ID NO: 24 - protein, 98 aa, synthetic
ASTKGPSVFPLAPSSKSTSGGTAALGCLVKDYFPEPVTVSWNSGALTSGVHTFPAVLQSSGLYSLSSVVTVPSSSLGTQTYICNVNHKPSNTKVDKKV

SEQ ID NO: 25 - protein, 107 aa, synthetic [sequence omitted]

SEQ ID NO: 26 - protein, 441 aa, synthetic
QVQLQQPGAELVKPGTSVKLSCKASGYPFTNYWMHWVRQRPGQGLEWIGEINPSNGRTNYNEKFKSLATLTLDKSSSTAYMHLNSLTSEDSAVYYCARGFAYWGQGTLVTVSSASTKGPSVFPLAPSSKSTSGGTAALGCLVKDYFPEPVTVSWNSGALTSGVHTFPAVLQSSGLYSLSSVVTVPSSSLGTQTYICNVNHKPSNTKVDKKVEPKSCDKTHTCPPCPAPELLGGPSVFLFPPKPKDTLMISRTPEVTCVVVDVSHEDPEVKFNWYVDGVEVHNAKTKPREEQYNSTYRVVSVLTVLHQDWLNGKEYKCKVSNKALPAPIEKTISKAKGQPREPQVYTLPPSRDELTKNQVSLTCLVKGFYPSDIAVEWESNGQPENNYKTTPPVLDSDGSFFLYSKLTVDKSRWQQGNVFSCSVMHEALHNHYTQKSLSLSP

SEQ ID NO: 27 - protein, 213 aa, synthetic
QIVLSQFPAIMSASPGEKVTMTCSASSSVSFMHWYQQKSGTSPKRWIYDTTKLASGVPARFTGSGSGTSYSLTISSMEAEDAATYYCQQWNSHPLTFGPGTKLELKRTVAAPSVFIFPPSDEQLKSGTASVVCLLNNFYPREAKVQWKVDNALQSGNSQESVTEQDSKDSTYSLSSTLTLSKADYEKHKVYACEVTHQGLSSPVTKSFNRGEC